European Patent Specification EP 4 093 403 B1, published September 30, 2026. Title: COMPOSITIONS FOR INHIBITION OF HERPESVIRUSES. Applicant: BOGER, Ravit. The sequence listing filed with the application follows.

SEQUENCE LISTING (3 sequences)

SEQ ID NO: 1 - DNA, 21 bp, Artificial Sequence
  Primer forward 5
gcgtgctttttagcctctgca

SEQ ID NO: 2 - DNA, 22 bp, Artificial Sequence
  Primer reverse 5
aaaagtttgtgccccaacggta

SEQ ID NO: 3 - DNA, 22 bp, Artificial Sequence
  US17 probe FAM 5'
tgatcgggcgttatcgcgttct